European Patent Application EP 4 707 382 A1, published March 11, 2026. Title: Method for producing metabolically activated liver organoid, composition, and method for evaluating test substance. Applicant: JSR Corporation. The sequence listing filed with the application follows.

SEQUENCE LISTING (14 sequences)

SEQ ID NO: 1 - DNA, 24 bp, Homo sapiens
  source 1..24: mol_type = other DNA
ctcatgaagatcagtgagcgctat

SEQ ID NO: 2 - DNA, 20 bp, Homo sapiens
  source 1..20: mol_type = other DNA
ctccccgttgctgaatacca

SEQ ID NO: 3 - DNA, 20 bp, Homo sapiens
  source 1..20: mol_type = other DNA
tatggaaaagtgtggggctt

SEQ ID NO: 4 - DNA, 21 bp, Homo sapiens
  source 1..21: mol_type = other DNA
tccggtttgtgaagacagaat

SEQ ID NO: 5 - DNA, 19 bp, Homo sapiens
  source 1..19: mol_type = other DNA
cgcgcacctctatggcatt

SEQ ID NO: 6 - DNA, 22 bp, Homo sapiens
  source 1..22: mol_type = other DNA
ttcttctgacacgagaacacac

SEQ ID NO: 7 - DNA, 20 bp, Homo sapiens
  source 1..20: mol_type = other DNA
aaaacggcctgaacctctcg

SEQ ID NO: 8 - DNA, 21 bp, Homo sapiens
  source 1..21: mol_type = other DNA
acacagctcagcgttattctc

SEQ ID NO: 9 - DNA, 19 bp, Homo sapiens
  source 1..19: mol_type = other DNA
tccgtggttctggcctaca

SEQ ID NO: 10 - DNA, 21 bp, Homo sapiens
  source 1..21: mol_type = other DNA
ggcttcctcgaagtcttcctt

SEQ ID NO: 11 - DNA, 22 bp, Homo sapiens
  source 1..22: mol_type = other DNA
aatgaggtgggcttaaagcaag

SEQ ID NO: 12 - DNA, 21 bp, Homo sapiens
  source 1..21: mol_type = other DNA
agttccactccacagttcaga

SEQ ID NO: 13 - DNA, 21 bp, Homo sapiens
  source 1..21: mol_type = other DNA
cagatgtgcaaggataagcgg

SEQ ID NO: 14 - DNA, 22 bp, Homo sapiens
  source 1..22: mol_type = other DNA
gcggtttggtcagataaaggtg